European Patent Application EP 4 166 010 A1, published April 19, 2023. Title: HIGH-PURITY STEVIOL GLYCOSIDES. Applicant: PureCircle SDN BHD. The sequence listing filed with the application follows.

SEQUENCE LISTING (13 sequences)

SEQ ID NO: 1 - DNA, 1397 bp, Stevia rebaudiana
ccatggcccatatggaaaacaaaaccgaaaccaccgttcgtcgtcgtcgccgtattattctgtttccggttccgtttcagggtcatattaatccgattctgcagctggcaaatgtgctgtatagcaaaggttttagcattaccatttttcataccaattttaacaaaccgaaaaccagcaattatccgcattttacctttcgctttattctggataatgatccgcaggatgaacgcattagcaatctgccgacacatggtccgctggcaggtatgcgtattccgattattaacgaacatggtgcagatgaactgcgtcgtgaactggaactgctgatgctggcaagcgaagaagatgaagaagttagctgtctgattaccgatgcactgtggtattttgcacagagcgttgcagatagcctgaatctgcgtcgtctggttctgatgaccagcagcctgtttaactttcatgcacatgttagcctgccgcagtttgatgaactgggttatctggatccggatgataaaacccgtctggaagaacaggcaagcggttttccgatgctgaaagtgaaagatatcaaaagcgcctatagcaattggcagattctgaaagaaattctgggcaaaatgattaaacagaccaaagcaagcagcggtgttatttggaatagctttaaagaactggaagaaagcgaactggaaaccgtgattcgtgaaattccggcaccgagctttctgattccgctgccgaaacatctgaccgcaagcagcagcagcctgctggatcatgatcgtaccgtttttcagtggctggatcagcagcctccgagcagcgttctgtatgttagctttggtagcaccagcgaagttgatgaaaaagattttctggaaattgcccgtggtctggttgatagcaaacagagctttctgtgggttgttcgtccgggttttgttaaaggtagcacctgggttgaaccgctgccggatggttttctgggtgaacgtggtcgtattgttaaatgggttccgcagcaagaagttctggcacacggcgcaattggtgcattttggacccatagcggttggaatagcaccctggaaagcgtttgtgaaggtgttccgatgatttttagcgattttggtctggatcagccgctgaatgcacgttatatgagtgatgttctgaaagtgggtgtgtatctggaaaatggttgggaacgtggtgaaattgcaaatgcaattcgtcgtgttatggtggatgaagaaggtgaatatattcgtcagaatgcccgtgttctgaaacagaaagcagatgttagcctgatgaaaggtggtagcagctatgaaagcctggaaagtctggttagctatattagcagcctgtaataactcgag

SEQ ID NO: 2 - DNA, 1442 bp, Stevia rebaudiana
ccatggcacatatggcaaccagcgatagcattgttgatgatcgtaaacagctgcatgttgcaacctttccgtggctggcatttggtcatattctgccgtatctgcagctgagcaaactgattgcagaaaaaggtcataaagtgagctttctgagcaccacccgtaatattcagcgtctgagcagccatattagtccgctgattaatgttgttcagctgaccctgcctcgtgttcaagaactgccggaagatgccgaagcaaccaccgatgttcatccggaagatattccgtatctgaaaaaagcaagtgatggtctgcagccggaagttacccgttttctggaacagcatagtccggattggatcatctatgattatacccattattggctgccgagcattgcagcaagcctgggtattagccgtgcacattttagcgttaccaccccgtgggcaattgcatatatgggtccgagcgcagatgcaatgattaatggtagtgatggtcgtaccaccgttgaagatctgaccacccctccgaaatggtttccgtttccgaccaaagtttgttggcgtaaacatgatctggcacgtctggttccgtataaagcaccgggtattagtgatggttatcgtatgggtctggttctgaaaggtagcgattgtctgctgagcaaatgctatcatgaatttggcacccagtggctgccgctgctggaaaccctgcatcaggttccggttgttccggtgggtctgctgcctccggaagttccgggtgatgaaaaagatgaaacctgggttagcatcaaaaaatggctggatggtaaacagaaaggtagcgtggtttatgttgcactgggtagcgaagttctggttagccagaccgaagttgttgaactggcactgggtctggaactgagcggtctgccgtttgtttgggcatatcgtaaaccgaaaggtccggcaaaaagcgatagcgttgaactgccggatggttttgttgaacgtacccgtgatcgtggtctggtttggaccagctgggcacctcagctgcgtattctgagccatgaaagcgtttgtggttttctgacccattgtggtagcggtagcattgtggaaggtctgatgtttggtcatccgctgattatgctgccgatttttggtgatcagccgctgaatgcacgtctgctggaagataaacaggttggtattgaaattccgcgtaatgaagaagatggttgcctgaccaaagaaagcgttgcacgtagcctgcgtagcgttgttgttgaaaaagaaggcgaaatctataaagccaatgcacgtgaactgagcaaaatctataatgataccaaagtggaaaaagaatatgtgagccagttcgtggattatctggaaaaaaacacccgtgcagttgccattgatcacgaaagctaatgactcgag

SEQ ID NO: 3 - protein, 472 aa, Oryza sativa
MDDAHSSQSPLHVVIFPWLAFGHLLPCLDLAERLAARGHRVSFVSTPRNLARLPPVRPELAELVDLVALPLPRVDGLPDGAEATSDVPFDKFELHRKAFDGLAAPFSAFLDTACAGGKRPDWVLADLMHHWVALASQERGVPCAMILPCSAAVVASSAPPTESSADQREAIVRSMGTAAPSFEAKRATEEFATEGASGVSIMTRYSLTLQRSKLVAMRSCPELEPGAFTILTRFYGKPVVPFGLLPPRPDGARGVSKNGKHDAIMQWLDAQPAKSVVYVALGSEAPMSADLLRELAHGLDLAGTRFLWAMRKPAGVDADSVLPAGFLGRTGERGLVTTRWAPQVSILAHAAVCAFLTHCGWGSVVEGLQFGHPLIMLPILGDQGPNARILEGRKLGVAVPRNDEDGSFDRGGVAGAVRAVVVEEEGKTFFANARKLQEIVADREREERCIDEFVQHLTSWNELKNNSDGQYP

SEQ ID NO: 4 - protein, 502 aa, Avena strigosa
MAVKDEQQSPLHILLFPFLAPGHLIPIADMAALFASRGVRCTILTTPVNAAIIRSAVDRANDAFRGSDCPAIDISVVPFPDVGLPPGVENGNALTSPADRLKFFQAVAELREPFDRFLADNHPDAVVSDSFFHWSTDAAAEHGVPRLGFLGSSMFAGSCNESTLHNNPLETAADDPDALVSLPGLPHRVELRRSQMMDPKKRPDHWALLESVNAADQKSFGEVFNSFHELEPDYVEHYQTTLGRRTWLVGPVALASKDMAGRGSTSARSPDADSCLRWLDTKQPGSVVYVSFGTLIRFSPAELHELARGLDLSGKNFVWVLGRAGPDSSEWMPQGFADLITPRGDRGFIIRGWAPQMLILNHRALGGFVTHCGWNSTLESVSAGVPMVTWPRFADQFQNEKLIVEVLKVGVSIGAKDYGSGIENHDVIRGEVIAESIGKLMGSSEESDAIQRKAKDLGAEARSAVENGGSSYNDVGRLMDELMARRSSVKVGEDIIPTNDGL

SEQ ID NO: 5 - protein, 470 aa, Solanum lycopersicum
MSPKLHKELFFHSLYKKTRSNHTMATLKVLMFPFLAYGHISPYLNVAKKLADRGFLIYFCSTPINLKSTIEKIPEKYADSIHLIELHLPELPQLPPHYHTTNGLPPNLNQVLQKALKMSKPNFSKILQNLKPDLVIYDILQRWAKHVANEQNIPAVKLLTSGAAVFSYFFNVLKKPGVEFPFPGIYLRKIEQVRLSEMMSKSDKEKELEDDDDDDDLLVDGNMQIMLMSTSRTIEAKYIDFCTALTNWKVVPVGPPVQDLITNDVDDMELIDWLGTKDENSTVFVSFGSEYFLSKEDMEEVAFALELSNVNFIWVARFPKGEERNLEDALPKGFLERIGERGRVLDKFAPQPRILNHPSTGGFISHCGWNSAMESIDFGVPIIAMPMHLDQPMNARLIVELGVAVEIVRDDDGKIHRGEIAETLKGVITGKTGEKLRAKVRDISKNLKTIRDEEMDAAAEELIQLCRNGN

SEQ ID NO: 6 - protein, 464 aa, Oryza sativa
MHVVMLPWLAFGHILPFAEFAKRVARQGHRVTLFSTPRNTRRLIDVPPSLAGRIRVVDIPLPRVEHLPEHAEATIDLPSNDLRPYLRRAYDEAFSRELSRLLQETGPSRPDWVLADYAAYWAPAAASRHGVPCAFLSLFGAAALCFFGPAETLQGRGPYAKTEPAHLTAVPEYVPFPTTVAFRGNEARELFKPSLIPDESGVSESYRFSQSIEGCQLVAVRSNQEFEPEWLELLGELYQKPVIPIGMFPPPPPQDVAGHEETLRWLDRQEPNSVVYAAFGSEVKLTAEQLQRIALGLEASELPFIWAFRAPPDAGDGDGLPGGFKERVNGRGVVCRGWVPQVKFLAHASVGGFLTHAGWNSIAEGLANGVRLVLLPLMFEQGLNARQLAEKKVAVEVARDEDDGSFAANDIVDALRRVMVGEEGDEFGVKVKELAKVFGDDEVNDRYVRDFLKCLSEYKMQRQG

SEQ ID NO: 7 - protein, 515 aa, Arabidopsis lyrata
MDDKKEEVMHIAMFPWLAMGHLLPFLRLSKLLAQKGHKISFISTPRNILRLPKLPSNLSSSITFVSFPLPSISGLPPSSESSMDVPYNKQQSLKAAFDLLQPPLTEFLRLSSPDWIIYDYASHWLPSIAKELGISKAFFSLFNAATLCFMGPSSSLIEESRSTPEDFTVVPPWVPFKSTIVFRYHEVSRYVEKTDEDVTGVSDSVRFGYTIDGSDAVFVRSCPEFEPEWFSLLQDLYRKPVFPIGFLPPVIEDDDDDTTWVRIKEWLDKQRVNSVVYVSLGTEASLRREELTELALGLEKSETPFFWVLRNEPQIPDGFEERVKGRGMVHVGWVPQVKILSHESVGGFLTHCGWNSVVEGIGFGKVPIFLPVLNEQGLNTRLLQGKGLGVEVLRDERDGSFGSDSVADSVRLVMIDDAGEEIREKVKLMKGLFGNMDENIRYVDELVGFMRNDESSQLKEEEEEDDCSDDQSSEVSSETDEKELNLDLKEEKRRISVYKSLSSEFDDYVANEKMG

SEQ ID NO: 8 - protein, 772 aa, Oryza sativa
MHVVICPLLAFGHLLPCLDLAQRLACGHRVSFVSTPRNISRLPPVRPSLAPLVSFVALPLPRVEGLPNGAESTHNVPHDRPDMVELHLRAFDGLAAPFSEFLGTACADWVMPTSSAPRQTLSSNIHRNSSRPGTPAPSGRLLCPITPHSNTLERAAEKLVRSSRQNARARSLLAFTSPPLPYRDVFRSLLGLQMGRKQLNIAHETNGRRTGTLPLNLCRWMWKQRRCGKLRPSDVEFNTSRSNEAISPIGASLVNLQSIQSPNPRAVLPIASSGVRAVFIGRARTSTPTPPHAKPARSAAPRAHRPPSSVMDSGYSSSYAAAAGMHVVICPWLAFGHLLPCLDLAQRLASRGHRVSFVSTPRNISRLPPVRPALAPLVAFVALPLPRVEGLPDGAESTNDVPHDRPDMVELHRRAFDGLAAPFSEFLGTACADWVIVDVFHHWAAAAALEHKVPCAMMLLGSAHMIASIADRRLERAETESPAAAGQGRPAAAPTFEVARMKLIRTKGSSGMSLAERFSLTLSRSSLVVGRSCVEFEPETVPLLSTLRGKPITFLGLMPPLHEGRREDGEDATVRWLDAQPAKSVVYVALGSEVPLGVEKVHELALGLELAGTRFLWALRKPTGVSDADLLPAGFEERTRGRGVVATRWVPQMSILAHAAVGAFLTHCGWNSTIEGLMFGHPLIMLPIFGDQGPNARLIEAKNAGLQVARNDGDGSFDREGVAAAIRAVAVEEESSKVFQAKAKKLQEIVADMACHERYIDGFIQQLRSYKD

SEQ ID NO: 9 - protein, 442 aa, Solanum lycopersicum
MATNLRVLMFPWLAYGHISPFLNIAKQLADRGFLIYLCSTRINLESIIKKIPEKYADSIHLIELQLPELPELPPHYHTTNGLPPHLNPTLHKALKMSKPNFSRILQNLKPDLLIYDVLQPWAEHVANEQNIPAGKLLTSCAAVFSYFFSFRKNPGVEFPFPAIHLPEVEKVKIREILAKEPEEGGRLDEGNKQMMLMCTSRTIEAKYIDYCTELCNWKVVPVGPPFQDLITNDADNKELIDWLGTKHENSTVFVSFGSEYFLSKEDMEEVAFALELSNVNFIWVARFPKGEERNLEDALPKGFLERIGERGRVLDKFAPQPRILNHPSTGGFISHCGWNSAMESIDFGVPIIAMPIHNDQPINAKLMVELGVAVEIVRDDDGKIHRGEIAETLKSVVTGETGEILRAKVREISKNLKSIRDEEMDAVAEELIQLCRNSNKSK

SEQ ID NO: 10 - protein, 454 aa, Escherichia coli
MGTEVTVHKNTLRVLMFPWLAYGHISPFLNVAKKLVDRGFLIYLCSTAINLKSTIKKIPEKYSDSIQLIELHLPELPELPPHYHTTNGLPPHLNHTLQKALKMSKPNFSKILQNLKPDLVIYDLLQQWAEGVANEQNIPAVKLLTSGAAVLSYFFNLVKKPGVEFPFPAIYLRKNELEKMSELLAQSAKDKEPDGVDPFADGNMQVMLMSTSRIIEAKYIDYFSGLSNWKVVPVGPPVQDPIADDADEMELIDWLGKKDENSTVFVSFGSEYFLSKEDREEIAFGLELSNVNFIWVARFPKGEEQNLEDALPKGFLERIGDRGRVLDKFAPQPRILNHPSTGGFISHCGWNSVMESVDFGVPIIAMPIHLDQPMNARLIVELGVAVEIVRDDYGKIHREEIAEILKDVIAGKSGENLKAKMRDISKNLKSIRDEEMDTAAEELIQLCKNSPKLK

SEQ ID NO: 11 - protein, 458 aa, Stevia rebaudiana
MENKTETTVRRRRRIILFPVPFQGHINPILQLANVLYSKGFSITIFHTNFNKPKTSNYPHFTFRFILDNDPQDERISNLPTHGPLAGMRIPIINEHGADELRRELELLMLASEEDEEVSCLITDALWYFAQSVADSLNLRRLVLMTSSLFNFHAHVSLPQFDELGYLDPDDKTRLEEQASGFPMLKVKDIKSAYSNWQILKEILGKMIKQTKASSGVIWNSFKELEESELETVIREIPAPSFLIPLPKHLTASSSSLLDHDRTVFQWLDQQPPSSVLYVSFGSTSEVDEKDFLEIARGLVDSKQSFLWVVRPGFVKGSTWVEPLPDGFLGERGRIVKWVPQQEVLAHGAIGAFWTHSGWNSTLESVCEGVPMIFSDFGLDQPLNARYMSDVLKVGVYLENGWERGEIANAIRRVMVDEEGEYIRQNARVLKQKADVSLMKGGSSYESLESLVSYISSL

SEQ ID NO: 12 - protein, 470 aa, Solanum lycopersicum; identical to SEQ ID NO: 5

SEQ ID NO: 13 - protein, 808 aa, Arabidopsis thaliana
MANAERMITRVHSQRERLNETLVSERNEVLALLSRVEAKGKGILQQNQIIAEFEALPEQTRKKLEGGPFFDLLKSTQEAIVLPPWVALAVRPRPGVWEYLRVNLHALVVEELQPAEFLHFKEELVDGVKNGNFTLELDFEPFNASIPRPTLHKYIGNGVDFLNRHLSAKLFHDKESLLPLLKFLRLHSHQGKNLMLSEKIQNLNTLQHTLRKAEEYLAELKSETLYEEFEAKFEEIGLERGWGDNAERVLDMIRLLLDLLEAPDPCTLETFLGRVPMVFNVVILSPHGYFAQDNVLGYPDTGGQVVYILDQVRALEIEMLQRIKQQGLNIKPRILILTRLLPDAVGTTCGERLERVYDSEYCDILRVPFRTEKGIVRKWISRFEVWPYLETYTEDAAVELSKELNGKPDLIIGNYSDGNLVASLLAHKLGVTQCTIAHALEKTKYPDSDIYWKKLDDKYHFSCQFTADIFAMNHTDFIITSTFQEIAGSKETVGQYESHTAFTLPGLYRVVHGIDVFDPKFNIVSPGADMSIYFPYTEEKRRLTKFHSEIEELLYSDVENKEHLCVLKDKKKPILFTMARLDRVKNLSGLVEWYGKNTRLRELANLVVVGGDRRKESKDNEEKAEMKKMYDLIEEYKLNGQFRWISSQMDRVRNGELYRYICDTKGAFVQPALYEAFGLTVVEAMTCGLPTFATCKGGPAEIIVHGKSGFHIDPYHGDQAADTLADFFTKCKEDPSHWDEISKGGLQRIEEKYTWQIYSQRLLTLTGVYGFWKHVSNLDRLEARRYLEMFYALKYRPLAQAVPLAQDD